European Patent Specification EP 3 352 798 B1, published November 19, 2025. Title: A method for high level and stable gene transfer in lymphocytes. Applicant: Julius-Maximilians-Universität Würzburg. The sequence listing filed with the application follows.

SEQUENCE LISTING (24 sequences)

SEQ ID NO: 1 - DNA, 36 bp, Artificial Sequence
  L(+) primer
gtaatacgactcactatagggctccgcttaagggac

SEQ ID NO: 2 - DNA, 17 bp, Artificial Sequence
  L(-)FspBI primer
  misc_feature (17)..(17): n is g-AMINO
tagtcccttaagcggan

SEQ ID NO: 3 - DNA, 19 bp, Artificial Sequence
  Nested primer
agggctccgcttaagggac

SEQ ID NO: 4 - DNA, 22 bp, Artificial Sequence
  Linker primer
gtaatacgactcactatagggc

SEQ ID NO: 5 - DNA, 27 bp, Artificial Sequence
  T_Bal rev primer
gaattgtgatacagtgaattataagtg

SEQ ID NO: 6 - DNA, 27 bp, Artificial Sequence
  T_Bal primer
cttgtgtcatgcacaaagtagatgtcc

SEQ ID NO: 7 - DNA, 36 bp, Artificial Sequence
  T_Bal_long primer
cttgtgtcatgcacaaagtagatgtcctaactgact

SEQ ID NO: 8 - DNA, 25 bp, Artificial Sequence
  LAM_SB_50 primer
agttttaatgactccaacttaagtg

SEQ ID NO: 9 - DNA, 89 bp, Artificial Sequence
  SB20h-bc-ill-N primer
  misc_feature (59)..(64): nnnnnn is a TRUSEQ-ILLUMINA-INDEX barcode DNA sequence
aatgatacggcgaccaccgagatctacactctttccctacacgacgctcttccgatctnnnnnncttaagtgtatgtaaacttccgact

SEQ ID NO: 10 - DNA, 64 bp, Artificial Sequence
  PE-nest-ind1-N primer
  misc_feature (25)..(30): nnnnnn is a reverse complement DNA sequence of a TRUSEQ-ILLUMINA-INDEX sequence
caagcagaagacggcatacgagatnnnnnngtgactggagttcagacgtgtgctcttccgatct

SEQ ID NO: 11 - DNA, 59 bp, Artificial Sequence
  Linker_TruSeq_T+ primer
gtaatacgactcactatagggctccgcttaagggactcagacgtgtgctcttccgatct

SEQ ID NO: 12 - DNA, 17 bp, Artificial Sequence
  Linker_TruSeq_T- primer
  misc_feature (17)..(17): n is g-AMINO
gatcggaagagcacacn

SEQ ID NO: 13 - DNA, 64 bp, Artificial Sequence
  PE_NEST_IND6 primer
caagcagaagacggcatacgagatattggcgtgactggagttcagacgtgtgctcttccgatct

SEQ ID NO: 14 - DNA, 64 bp, Artificial Sequence
  PE_NEST_IND7 primer
caagcagaagacggcatacgagatagtctggtgactggagttcagacgtgtgctcttccgatct

SEQ ID NO: 15 - DNA, 64 bp, Artificial Sequence
  PE_NEST_IND8 primer
caagcagaagacggcatacgagattcaagtgtgactggagttcagacgtgtgctcttccgatct

SEQ ID NO: 16 - DNA, 20 bp, Artificial Sequence
  CAR-Fwd primer
atctggatgtcggggatcag

SEQ ID NO: 17 - DNA, 20 bp, Artificial Sequence
  CAR-probe oligonucleotide
  misc_feature (1)..(1): n is FAM-A
  misc_feature (20)..(20): n is T-BH1
ngcagcatggtggcggcgcn

SEQ ID NO: 18 - DNA, 20 bp, Artificial Sequence
  CAR-Rev primer
gcttgctcaactctacgtct

SEQ ID NO: 19 - DNA, 18 bp, Artificial Sequence
  MC-Fwd primer
ccgaccttaatgcgcctc

SEQ ID NO: 20 - DNA, 27 bp, Artificial Sequence
  MC-probe oligonucleotide
  misc_feature (1)..(1): n is FAM-G
  misc_feature (27)..(27): n is T-BH1
ncgctgtagcctcacgcccacatatgn

SEQ ID NO: 21 - DNA, 25 bp, Artificial Sequence
  MC-Rev primer
aggattaaatgtcaggaattgtgaa

SEQ ID NO: 22 - DNA, 20 bp, Artificial Sequence
  RPP30-Fwd primer
ggttaactacagctcccagc

SEQ ID NO: 23 - DNA, 24 bp, Artificial Sequence
  RPP30-probe oligonucleotide
  misc_feature (1)..(1): n is HEX-T
  misc_feature (24)..(24): n is C-BH1
nggacctgcgagcgggttctgacn

SEQ ID NO: 24 - DNA, 18 bp, Artificial Sequence
  RPP30-Rev primer
ctgtctccacaagtccgc